European Patent Application EP 4 122 447 A1, published January 25, 2023. Title: FUSION PROTEIN PREPARATION COMPRISING IL-2 AND CD80 PROTEINS. Applicant: GI Innovation, Inc. The sequence listing filed with the application follows.

SEQUENCE LISTING (38 sequences)

SEQ ID NO: 1 - protein, 25 aa, Artificial Sequence
  signal peptide (TPA)
MDAMLRGLCCVLLLCGAVFVSPSHA

SEQ ID NO: 2 - protein, 208 aa, Artificial Sequence [sequence omitted]

SEQ ID NO: 3 - protein, 30 aa, Artificial Sequence
  hinge with linker
GSGGGGSGGGGSGGGGSAESKYGPPCPPCP

SEQ ID NO: 4 - protein, 216 aa, Artificial Sequence
  immunoglobulin fc
APEAAGGPSVFLFPPKPKDQLMISRTPEVTCVVVDVSQEDPEVQFNWYVDGVEVHNAKTKPREEQFNSTYRVVSVLTVLHQDWLNGKEYKCKVSNKGLPSSIEKTISKAKGQPREPQVYTLPPSQEEMTKNQVSLTCLVKGFYPSDIAVEWESNGQPENNYKTTPPVLDSDGSFFLYSRLTVDKSRWQEGNVFSCSVLHEALHNHYTQKSLSLSLG

SEQ ID NO: 5 - protein, 5 aa, Artificial Sequence
  linker
GGGGS

SEQ ID NO: 6 - protein, 133 aa, Artificial Sequence
  hIL-2M
APTSSSTKKTQLQLEHLLLDLQMILNGINNYKNPKLTAMLTAKFYMPKKATELKHLQCLEEELKPLEEVLNLAQSKNFHLRPRDLISNINVIVLELKGSETTFMCEYADETATIVEFLNRWITFCQSIISTLT

SEQ ID NO: 7 - protein, 617 aa, Artificial Sequence
  fusion protein comprising variants of IL-2 and fragments of CD80
MDAMLRGLCCVLLLCGAVFVSPSHAVIHVTKEVKEVATLSCGHNVSVEELAQTRIYWQKEKKMVLTMMSGDMNIWPEYKNRTIFDITNNLSIVILALRPSDEGTYECVVLKYEKDAFKREHLAEVTLSVKADFPTPSISDFEIPTSNIRRIICSTSGGFPEPHLSWLENGEELNAINTTVSQDPETELYAVSSKLDFNMTTNHSFMCLIKYGHLRVNQTFNWNTTKQEHFPDNGSGGGGSGGGGSGGGGSAESKYGPPCPPCPAPEAAGGPSVFLFPPKPKDQLMISRTPEVTCVVVDVSQEDPEVQFNWYVDGVEVHNAKTKPREEQFNSTYRVVSVLTVLHQDWLNGKEYKCKVSNKGLPSSIEKTISKAKGQPREPQVYTLPPSQEEMTKNQVSLTCLVKGFYPSDIAVEWESNGQPENNYKTTPPVLDSDGSFFLYSRLTVDKSRWQEGNVFSCSVLHEALHNHYTQKSLSLSLGGGGGSAPTSSSTKKTQLQLEHLLLDLQMILNGINNYKNPKLTAMLTAKFYMPKKATELKHLQCLEEELKPLEEVLNLAQSKNFHLRPRDLISNINVIVLELKGSETTFMCEYADETATIVEFLNRWITFCQSIISTLT

SEQ ID NO: 8 - DNA, 1857 bp, Artificial Sequence
  nucleotiedes coding fusion protein (GI101)
atggatgctatgctgagaggcctgtgttgcgtgctgctgctgtgtggcgctgtgttcgtgtctccttctcacgctgtgatccacgtgaccaaagaagtgaaagaggtcgccacactgtcctgcggccacaacgtttcagtggaagaactggcccagaccaggatctactggcagaaagaaaagaaaatggtgctgaccatgatgtccggcgacatgaacatctggcctgagtacaagaaccggaccatcttcgacatcaccaacaacctgtccatcgtgattctggccctgaggccttctgatgagggcacctatgagtgcgtggtgctgaagtacgagaaggacgccttcaagcgcgagcacctggctgaagtgacactgtccgtgaaggccgactttcccacaccttccatctccgacttcgagatccctacctccaacatccggcggatcatctgttctacctctggcggctttcctgagcctcacctgtcttggctggaaaacggcgaggaactgaacgccatcaacaccaccgtgtctcaggaccccgaaaccgagctgtacgctgtgtcctccaagctggacttcaacatgaccaccaaccacagcttcatgtgcctgattaagtacggccacctgagagtgaaccagaccttcaactggaacaccaccaagcaagagcacttccctgacaatggatctggcggcggaggttctggcggaggtggaagcggaggcggaggatctgctgagtctaagtatggccctccttgtcctccatgtcctgctccagaagctgctggcggaccctctgtgttcctgtttcctccaaagcctaaggaccagctcatgatctctcggacacccgaagtgacctgcgtggtggtggatgtgtctcaagaggaccctgaggtgcagttcaattggtacgtggacggcgtggaagtgcacaacgccaagaccaagcctagagaggaacagttcaactccacctacagagtggtgtccgtgctgaccgtgctgcaccaggattggctgaacggcaaagagtacaagtgcaaggtgtccaacaagggcctgccttccagcatcgaaaagaccatctccaaggctaagggccagcctagggaaccccaggtttacaccctgcctccaagccaagaggaaatgaccaagaaccaggtgtccctgacctgcctggtcaagggcttctacccttccgacattgccgtggaatgggagtccaatggccagcctgagaacaactacaagaccacacctcctgtgctggactccgacggctccttctttctgtactctcgcctgaccgtggacaagtctagatggcaagagggcaacgtgttctcctgctctgtgctgcacgaggccctgcacaatcactacacccagaagtccctgtctctgtctcttggaggtggtggcggttctgcccctaccagctcctctaccaagaaaacccagctccagttggagcatctgctgctggacctccagatgattctgaacgggatcaacaactataagaaccccaagctgaccgccatgctgaccgctaagttctacatgcccaagaaggccaccgagctgaagcacctccagtgcctggaagaagaactgaagcccctggaagaggtgctgaatctggcccagtccaagaacttccacctgaggccacgggacctgatcagcaacatcaacgtgatcgtgctggaactgaagggctccgagacaacctttatgtgcgagtacgccgacgagacagccaccatcgtggaatttctgaaccggtggatcaccttctgccagagcatcatctccacactgacctgatga

SEQ ID NO: 9 - protein, 592 aa, Artificial Sequence
  fusion protein (GI101)
VIHVTKEVKEVATLSCGHNVSVEELAQTRIYWQKEKKMVLTMMSGDMNIWPEYKNRTIFDITNNLSIVILALRPSDEGTYECVVLKYEKDAFKREHLAEVTLSVKADFPTPSISDFEIPTSNIRRIICSTSGGFPEPHLSWLENGEELNAINTTVSQDPETELYAVSSKLDFNMTTNHSFMCLIKYGHLRVNQTFNWNTTKQEHFPDNGSGGGGSGGGGSGGGGSAESKYGPPCPPCPAPEAAGGPSVFLFPPKPKDQLMISRTPEVTCVVVDVSQEDPEVQFNWYVDGVEVHNAKTKPREEQFNSTYRVVSVLTVLHQDWLNGKEYKCKVSNKGLPSSIEKTISKAKGQPREPQVYTLPPSQEEMTKNQVSLTCLVKGFYPSDIAVEWESNGQPENNYKTTPPVLDSDGSFFLYSRLTVDKSRWQEGNVFSCSVLHEALHNHYTQKSLSLSLGGGGGSAPTSSSTKKTQLQLEHLLLDLQMILNGINNYKNPKLTAMLTAKFYMPKKATELKHLQCLEEELKPLEEVLNLAQSKNFHLRPRDLISNINVIVLELKGSETTFMCEYADETATIVEFLNRWITFCQSIISTLT

SEQ ID NO: 10 - protein, 133 aa, Artificial Sequence [sequence omitted]

SEQ ID NO: 11 - protein, 288 aa, Artificial Sequence
  CD80
MGHTRRQGTSPSKCPYLNFFQLLVLAGLSHFCSGVIHVTKEVKEVATLSCGHNVSVEELAQTRIYWQKEKKMVLTMMSGDMNIWPEYKNRTIFDITNNLSIVILALRPSDEGTYECVVLKYEKDAFKREHLAEVTLSVKADFPTPSISDFEIPTSNIRRIICSTSGGFPEPHLSWLENGEELNAINTTVSQDPETELYAVSSKLDFNMTTNHSFMCLIKYGHLRVNQTFNWNTTKQEHFPDNLLPSWAITLISVNGIFVICCLTYCFAPRCRERRRNERLRRESVRPV

SEQ ID NO: 12 - protein, 215 aa, Artificial Sequence
  modified Fc
SHTQPLGVFLFPPKPKDTLMISRTPEVTCVVVDVSQEDPEVQFNWYVDGVEVHNAKTKPREEQFNSTYRVVSVLTVLHQDWLNGKEYKCKVSNKGLPSSIEKTISKAKGQPREPQVYTLPPSQEEMTKNQVSLTCLVKGFYPSDIAVEWESNGQPENNYKTTPPVLDSDGSFFLYSRLTVDKSRWQEGNVFSCSVMHEALHNHYTQKSLSLSLGK

SEQ ID NO: 13 - protein, 306 aa, Artificial Sequence
  mCD80
MACNCQLMQDTPLLKFPCPRLILLFVLLIRLSQVSSDVDEQLSKSVKDKVLLPCRYNSPHEDESEDRIYWQKHDKVVLSVIAGKLKVWPEYKNRTLYDNTTYSLIILGLVLSDRGTYSCVVQKKERGTYEVKHLALVKLSIKADFSTPNITESGNPSADTKRITCFASGGFPKPRFSWLENGRELPGINTTISQDPESELYTISSQLDFNTTRNHTIKCLIKYGDAHVSEDFTWEKPPEDPPDSKNTLVLFGAGFGAVITVVVIVVIIKCFCKHRSCFRRNEASRETNNSLTFGPEEALAEQTVFL

SEQ ID NO: 14 - DNA, 1848 bp, Artificial Sequence
  nucleotiedes coding fusion protein (mGI101)
atggatgctatgctgagaggcctgtgttgcgtgctgctgctgtgtggcgctgtgttcgtgtctccttctcacgctgtggacgagcagctctccaagtccgtgaaggataaggtcctgctgccttgccggtacaactctcctcacgaggacgagtctgaggaccggatctactggcagaaacacgacaaggtggtgctgtccgtgatcgccggaaagctgaaagtgtggcctgagtacaagaacaggaccctgtacgacaacaccacctacagcctgatcatcctgggcctcgtgctgagcgatagaggcacctattcttgcgtggtgcagaagaaagagcggggcacctacgaagtgaagcacctggctctggtcaagctgtccatcaaggccgacttcagcacccctaacatcaccgagtctggcaacccttccgccgacaccaagagaatcacctgtttcgcctctggcggcttccctaagcctcggttctcttggctggaaaacggcagagagctgcccggcatcaataccaccatttctcaggacccagagtccgagctgtacaccatctccagccagctcgactttaacaccaccagaaaccacaccatcaagtgcctgattaagtacggcgacgcccacgtgtccgaggactttacttgggagaaacctcctgaggaccctcctgactctggatctggcggcggaggttctggcggaggtggaagcggaggcggaggatctgctgagtctaagtatggccctccttgtcctccatgtcctgctccagaagctgctggcggaccctctgtgttcctgtttcctccaaagcctaaggaccagctcatgatctctcggacccctgaagtgacctgcgtggtggtggatgtgtctcaagaggaccctgaggtgcagttcaattggtacgtggacggcgtggaagtgcacaacgccaagaccaagcctagagaggaacagttcaactccacctatagagtggtgtccgtgctgaccgtgctgcaccaggattggctgaacggcaaagagtacaagtgcaaggtgtccaacaagggcctgccttccagcatcgaaaagaccatcagcaaggctaagggccagcctagggaaccccaggtttacaccctgcctccaagccaagaggaaatgaccaagaaccaggtgtccctgacctgcctggtcaagggcttctacccttccgacattgccgtggaatgggagtccaatggccagcctgagaacaactacaagaccacacctcctgtgctggactccgacggctccttctttctgtactctcgcctgaccgtggacaagtctaggtggcaagagggcaacgtgttctcctgctctgtgctgcacgaggctctgcacaaccactacacccagaagtccctgtctctgtctcttggaggtggtggcggttctgcccctacctccagctctaccaagaaaacccagctccagttggagcatctgctgctggacctccagatgatcctgaatggcatcaacaattacaagaaccccaagctgaccgccatgctgaccgctaagttctacatgcccaagaaggccaccgagctgaagcacttgcagtgcctggaagaggaactgaagcccctggaagaagtgctgaatctggcccagtccaagaacttccacctgaggcctagggacctgatctccaacatcaacgtgatcgtgctggaactgaaaggctccgagacaaccttcatgtgcgagtacgccgacgagacagccaccatcgtggaatttctgaaccggtggatcaccttctgccagagcatcatctccacactgacc

SEQ ID NO: 15 - protein, 616 aa, Artificial Sequence
  fusion protein (mGI101)
MDAMLRGLCCVLLLCGAVFVSPSHAVDEQLSKSVKDKVLLPCRYNSPHEDESEDRIYWQKHDKVVLSVIAGKLKVWPEYKNRTLYDNTTYSLIILGLVLSDRGTYSCVVQKKERGTYEVKHLALVKLSIKADFSTPNITESGNPSADTKRITCFASGGFPKPRFSWLENGRELPGINTTISQDPESELYTISSQLDFNTTRNHTIKCLIKYGDAHVSEDFTWEKPPEDPPDSGSGGGGSGGGGSGGGGSAESKYGPPCPPCPAPEAAGGPSVFLFPPKPKDQLMISRTPEVTCVVVDVSQEDPEVQFNWYVDGVEVHNAKTKPREEQFNSTYRVVSVLTVLHQDWLNGKEYKCKVSNKGLPSSIEKTISKAKGQPREPQVYTLPPSQEEMTKNQVSLTCLVKGFYPSDIAVEWESNGQPENNYKTTPPVLDSDGSFFLYSRLTVDKSRWQEGNVFSCSVLHEALHNHYTQKSLSLSLGGGGGSAPTSSSTKKTQLQLEHLLLDLQMILNGINNYKNPKLTAMLTAKFYMPKKATELKHLQCLEEELKPLEEVLNLAQSKNFHLRPRDLISNINVIVLELKGSETTFMCEYADETATIVEFLNRWITFCQSIISTLT

SEQ ID NO: 16 - DNA, 1437 bp, Artificial Sequence
  nucleotiedes coding fusion protein (GI101C1)
atggatgctatgctgagaggcctgtgttgcgtgctgctgctgtgtggcgctgtgttcgtgtctccttctcacgctgtgatccacgtgaccaaagaagtgaaagaggtcgccacactgtcctgcggccacaacgtttcagtggaagaactggcccagaccaggatctactggcagaaagaaaagaaaatggtgctgaccatgatgtccggcgacatgaacatctggcctgagtacaagaaccggaccatcttcgacatcaccaacaacctgtccatcgtgattctggccctgaggccttctgatgagggcacctatgagtgcgtggtgctgaagtacgagaaggacgccttcaagcgcgagcacctggctgaagtgacactgtccgtgaaggccgactttcccacaccttccatctccgacttcgagatccctacctccaacatccggcggatcatctgttctacctctggcggctttcctgagcctcacctgtcttggctggaaaacggcgaggaactgaacgccatcaacaccaccgtgtctcaggaccccgaaaccgagctgtacgctgtgtcctccaagctggacttcaacatgaccaccaaccacagcttcatgtgcctgattaagtacggccacctgagagtgaaccagaccttcaactggaacaccaccaagcaagagcacttccctgacaatggatctggcggcggaggttctggcggaggtggaagcggaggcggaggatctgctgagtctaagtatggccctccttgtcctccatgtcctgctccagaagctgctggcggaccctctgtgttcctgtttcctccaaagcctaaggaccagctcatgatctctcggacacccgaagtgacctgcgtggtggtggatgtgtctcaagaggaccctgaggtgcagttcaattggtacgtggacggcgtggaagtgcacaacgccaagaccaagcctagagaggaacagttcaactccacctacagagtggtgtccgtgctgaccgtgctgcaccaggattggctgaacggcaaagagtacaagtgcaaggtgtccaacaagggcctgccttccagcatcgaaaagaccatctccaaggctaagggccagcctagggaaccccaggtttacaccctgcctccaagccaagaggaaatgaccaagaaccaggtgtccctgacctgcctggtcaagggcttctacccttccgacattgccgtggaatgggagtccaatggccagcctgagaacaactacaagaccacacctcctgtgctggactccgacggctccttctttctgtactctcgcctgaccgtggacaagtctaggtggcaagagggcaacgtgttctcctgctctgtgctgcacgaggccctgcacaatcactacacccagaagtccctgtctctgtccctgggc

SEQ ID NO: 17 - protein, 454 aa, Artificial Sequence
  fusion protein (GI101C1)
VIHVTKEVKEVATLSCGHNVSVEELAQTRIYWQKEKKMVLTMMSGDMNIWPEYKNRTIFDITNNLSIVILALRPSDEGTYECVVLKYEKDAFKREHLAEVTLSVKADFPTPSISDFEIPTSNIRRIICSTSGGFPEPHLSWLENGEELNAINTTVSQDPETELYAVSSKLDFNMTTNHSFMCLIKYGHLRVNQTFNWNTTKQEHFPDNGSGGGGSGGGGSGGGGSAESKYGPPCPPCPAPEAAGGPSVFLFPPKPKDQLMISRTPEVTCVVVDVSQEDPEVQFNWYVDGVEVHNAKTKPREEQFNSTYRVVSVLTVLHQDWLNGKEYKCKVSNKGLPSSIEKTISKAKGQPREPQVYTLPPSQEEMTKNQVSLTCLVKGFYPSDIAVEWESNGQPENNYKTTPPVLDSDGSFFLYSRLTVDKSRWQEGNVFSCSVLHEALHNHYTQKSLSLSLG

SEQ ID NO: 18 - DNA, 1176 bp, Artificial Sequence
  nucleotiedes coding fusion protein (GI101C2)
atggatgctatgctgagaggcctgtgttgcgtgctgctgctgtgtggcgctgtgttcgtgtctccatctcacgccgctgagtctaagtacggccctccttgtcctccatgtcctgctccagaagctgctggcggaccctctgtgttcctgtttcctccaaagcctaaggaccagctcatgatctctcggacccctgaagtgacctgcgtggtggtggatgtgtctcaagaggaccctgaggtgcagttcaattggtacgtggacggcgtggaagtgcacaacgccaagaccaagcctagagaggaacagttcaactccacctacagagtggtgtccgtgctgaccgtgctgcaccaggattggctgaacggcaaagagtacaagtgcaaggtgtccaacaagggcctgccttccagcatcgaaaagaccatctccaaggctaagggccagcctagggaaccccaggtttacaccctgcctccaagccaagaggaaatgaccaagaaccaggtgtccctgacctgcctggtcaagggcttctacccttccgacattgccgtggaatgggagtccaatggccagcctgagaacaactacaagaccacacctcctgtgctggactccgacggctccttctttctgtactctcgcctgaccgtggacaagtctaggtggcaagagggcaacgtgttctcctgctctgtgctgcacgaggccctgcacaatcactacacccagaagtccctgtctctgtctcttggcggaggcggaggatctgctcctacctccagctccaccaagaaaacccagctccagttggagcatctgctgctggacctccagatgatcctgaatggcatcaacaattacaagaaccccaagctgaccgccatgctgaccgctaagttctacatgcccaagaaggccaccgagctgaagcacctccagtgcctggaagaggaactgaagcccctggaagaagtgctgaatctggcccagtccaagaacttccacctgaggcctagggacctgatctccaacatcaacgtgatcgtgctggaactgaaaggctccgagacaaccttcatgtgcgagtacgccgacgagacagccaccatcgtggaatttctgaaccggtggatcaccttctgccagtccatcatctccacactgacc

SEQ ID NO: 19 - protein, 367 aa, Artificial Sequence
  fusion protein (GI101C2)
AESKYGPPCPPCPAPEAAGGPSVFLFPPKPKDQLMISRTPEVTCVVVDVSQEDPEVQFNWYVDGVEVHNAKTKPREEQFNSTYRVVSVLTVLHQDWLNGKEYKCKVSNKGLPSSIEKTISKAKGQPREPQVYTLPPSQEEMTKNQVSLTCLVKGFYPSDIAVEWESNGQPENNYKTTPPVLDSDGSFFLYSRLTVDKSRWQEGNVFSCSVLHEALHNHYTQKSLSLSLGGGGGSAPTSSSTKKTQLQLEHLLLDLQMILNGINNYKNPKLTAMLTAKFYMPKKATELKHLQCLEEELKPLEEVLNLAQSKNFHLRPRDLISNINVIVLELKGSETTFMCEYADETATIVEFLNRWITFCQSIISTLT

SEQ ID NO: 20 - DNA, 1434 bp, Artificial Sequence
  nucleotiedes coding fusion protein (mGI101C1)
atggatgctatgctgagaggcctgtgttgcgtgctgctgctgtgtggcgctgtgttcgtgtctccttctcacgctgtggacgagcagctctccaagtccgtgaaggataaggtcctgctgccttgccggtacaactctcctcacgaggacgagtctgaggaccggatctactggcagaaacacgacaaggtggtgctgtccgtgatcgccggaaagctgaaagtgtggcctgagtacaagaacaggaccctgtacgacaacaccacctacagcctgatcatcctgggcctcgtgctgagcgatagaggcacctattcttgcgtggtgcagaagaaagagcggggcacctacgaagtgaagcacctggctctggtcaagctgtccatcaaggccgacttcagcacccctaacatcaccgagtctggcaacccttccgccgacaccaagagaatcacctgtttcgcctctggcggcttccctaagcctcggttctcttggctggaaaacggcagagagctgcccggcatcaataccaccatttctcaggacccagagtccgagctgtacaccatctccagccagctcgactttaacaccaccagaaaccacaccatcaagtgcctgattaagtacggcgacgcccacgtgtccgaggactttacttgggagaaacctcctgaggaccctcctgactctggatctggcggcggaggttctggcggaggtggaagcggaggcggaggatctgctgagtctaagtatggccctccttgtcctccatgtcctgctccagaagctgctggcggaccctctgtgttcctgtttcctccaaagcctaaggaccagctcatgatctctcggacccctgaagtgacctgcgtggtggtggatgtgtctcaagaggaccctgaggtgcagttcaattggtacgtggacggcgtggaagtgcacaacgccaagaccaagcctagagaggaacagttcaactccacctatagagtggtgtccgtgctgaccgtgctgcaccaggattggctgaacggcaaagagtacaagtgcaaggtgtccaacaagggcctgccttccagcatcgaaaagaccatcagcaaggctaagggccagcctagggaaccccaggtttacaccctgcctccaagccaagaggaaatgaccaagaaccaggtgtccctgacctgcctggtcaagggcttctacccttccgacattgccgtggaatgggagtccaatggccagcctgagaacaactacaagaccacacctcctgtgctggactccgacggctccttctttctgtactctcgcctgaccgtggacaagtctaggtggcaagagggcaacgtgttctcctgctctgtgctgcacgaggctctgcacaaccactacacccagaagtccctgtctctgtccctgggc

SEQ ID NO: 21 - protein, 478 aa, Artificial Sequence
  fusion protein (mGI101C1)
MDAMLRGLCCVLLLCGAVFVSPSHAVDEQLSKSVKDKVLLPCRYNSPHEDESEDRIYWQKHDKVVLSVIAGKLKVWPEYKNRTLYDNTTYSLIILGLVLSDRGTYSCVVQKKERGTYEVKHLALVKLSIKADFSTPNITESGNPSADTKRITCFASGGFPKPRFSWLENGRELPGINTTISQDPESELYTISSQLDFNTTRNHTIKCLIKYGDAHVSEDFTWEKPPEDPPDSGSGGGGSGGGGSGGGGSAESKYGPPCPPCPAPEAAGGPSVFLFPPKPKDQLMISRTPEVTCVVVDVSQEDPEVQFNWYVDGVEVHNAKTKPREEQFNSTYRVVSVLTVLHQDWLNGKEYKCKVSNKGLPSSIEKTISKAKGQPREPQVYTLPPSQEEMTKNQVSLTCLVKGFYPSDIAVEWESNGQPENNYKTTPPVLDSDGSFFLYSRLTVDKSRWQEGNVFSCSVLHEALHNHYTQKSLSLSLG

SEQ ID NO: 22 - protein, 133 aa, Artificial Sequence
  variants of IL-2 (3M, M45)
APTSSSTKKTQLQLEHLLLDLQMILNGINNYKNPKLTAMLTAKFAMPKKATELKHLQCLEEELKPLEEVLNLAQSKNFHLRPRDLISNINVIVLELKGSETTFMCEYADETATIVEFLNRWITFCQSIISTLT

SEQ ID NO: 23 - protein, 133 aa, Artificial Sequence
  variants of IL-2 (3M, M61)
APTSSSTKKTQLQLEHLLLDLQMILNGINNYKNPKLTAMLTAKFYMPKKATELKHLQCLERELKPLEEVLNLAQSKNFHLRPRDLISNINVIVLELKGSETTFMCEYADETATIVEFLNRWITFCQSIISTLT

SEQ ID NO: 24 - protein, 133 aa, Artificial Sequence
  variants of IL-2 (3M, M72)
APTSSSTKKTQLQLEHLLLDLQMILNGINNYKNPKLTAMLTAKFYMPKKATELKHLQCLEEELKPLEEVLNGAQSKNFHLRPRDLISNINVIVLELKGSETTFMCEYADETATIVEFLNRWITFCQSIISTLT

SEQ ID NO: 25 - DNA, 1851 bp, Artificial Sequence
  nucleotiedes coding fusion protein (GI102-M45)
atggatgctatgctgagaggcctgtgttgcgtgctgctgctgtgtggcgctgtgttcgtgtctccttctcacgctgtgatccacgtgaccaaagaagtgaaagaggtcgccacactgtcctgcggccacaacgtttcagtggaagaactggcccagaccaggatctactggcagaaagaaaagaaaatggtgctgaccatgatgtccggcgacatgaacatctggcctgagtacaagaaccggaccatcttcgacatcaccaacaacctgtccatcgtgattctggccctgaggccttctgatgagggcacctatgagtgcgtggtgctgaagtacgagaaggacgccttcaagcgcgagcacctggctgaagtgacactgtccgtgaaggccgactttcccacaccttccatctccgacttcgagatccctacctccaacatccggcggatcatctgttctacctctggcggctttcctgagcctcacctgtcttggctggaaaacggcgaggaactgaacgccatcaacaccaccgtgtctcaggaccccgaaaccgagctgtacgctgtgtcctccaagctggacttcaacatgaccaccaaccacagcttcatgtgcctgattaagtacggccacctgagagtgaaccagaccttcaactggaacaccaccaagcaagagcacttccctgacaatggatctggcggcggaggttctggcggaggtggaagcggaggcggaggatctgctgagtctaagtatggccctccttgtcctccatgtcctgctccagaagctgctggcggaccctctgtgttcctgtttcctccaaagcctaaggaccagctcatgatctctcggacacccgaagtgacctgcgtggtggtggatgtgtctcaagaggaccctgaggtgcagttcaattggtacgtggacggcgtggaagtgcacaacgccaagaccaagcctagagaggaacagttcaactccacctacagagtggtgtccgtgctgaccgtgctgcaccaggattggctgaacggcaaagagtacaagtgcaaggtgtccaacaagggcctgccttccagcatcgaaaagaccatctccaaggctaagggccagcctagggaaccccaggtttacaccctgcctccaagccaagaggaaatgaccaagaaccaggtgtccctgacctgcctggtcaagggcttctacccttccgacattgccgtggaatgggagtccaatggccagcctgagaacaactacaagaccacacctcctgtgctggactccgacggctccttctttctgtactctcgcctgaccgtggacaagtctagatggcaagagggcaacgtgttctcctgctctgtgctgcacgaggccctgcacaatcactacacccagaagtccctgtctctgtctcttggaggtggtggcggttctgcccctaccagctcctctaccaagaaaacccagctccagttggagcatctgctgctggacctccagatgattctgaacgggatcaacaactataagaaccccaagctgaccgccatgctgaccgctaagttcgccatgcccaagaaggccaccgagctgaagcacctccagtgcctggaagaagaactgaagcccctggaagaggtgctgaatctggcccagtccaagaacttccacctgaggccacgggacctgatcagcaacatcaacgtgatcgtgctggaactgaagggctccgagacaacctttatgtgcgagtacgccgacgagacagccaccatcgtggaatttctgaaccggtggatcaccttctgccagagcatcatctccacactgacc

SEQ ID NO: 26 - protein, 592 aa, Artificial Sequence
  fusion protein (GI102-M45)
VIHVTKEVKEVATLSCGHNVSVEELAQTRIYWQKEKKMVLTMMSGDMNIWPEYKNRTIFDITNNLSIVILALRPSDEGTYECVVLKYEKDAFKREHLAEVTLSVKADFPTPSISDFEIPTSNIRRIICSTSGGFPEPHLSWLENGEELNAINTTVSQDPETELYAVSSKLDFNMTTNHSFMCLIKYGHLRVNQTFNWNTTKQEHFPDNGSGGGGSGGGGSGGGGSAESKYGPPCPPCPAPEAAGGPSVFLFPPKPKDQLMISRTPEVTCVVVDVSQEDPEVQFNWYVDGVEVHNAKTKPREEQFNSTYRVVSVLTVLHQDWLNGKEYKCKVSNKGLPSSIEKTISKAKGQPREPQVYTLPPSQEEMTKNQVSLTCLVKGFYPSDIAVEWESNGQPENNYKTTPPVLDSDGSFFLYSRLTVDKSRWQEGNVFSCSVLHEALHNHYTQKSLSLSLGGGGGSAPTSSSTKKTQLQLEHLLLDLQMILNGINNYKNPKLTAMLTAKFAMPKKATELKHLQCLEEELKPLEEVLNLAQSKNFHLRPRDLISNINVIVLELKGSETTFMCEYADETATIVEFLNRWITFCQSIISTLT

SEQ ID NO: 27 - DNA, 1851 bp, Artificial Sequence
  nucleotiedes coding fusion protein (GI102-M61)
atggatgctatgctgagaggcctgtgttgcgtgctgctgctgtgtggcgctgtgttcgtgtctccttctcacgctgtgatccacgtgaccaaagaagtgaaagaggtcgccacactgtcctgcggccacaacgtttcagtggaagaactggcccagaccaggatctactggcagaaagaaaagaaaatggtgctgaccatgatgtccggcgacatgaacatctggcctgagtacaagaaccggaccatcttcgacatcaccaacaacctgtccatcgtgattctggccctgaggccttctgatgagggcacctatgagtgcgtggtgctgaagtacgagaaggacgccttcaagcgcgagcacctggctgaagtgacactgtccgtgaaggccgactttcccacaccttccatctccgacttcgagatccctacctccaacatccggcggatcatctgttctacctctggcggctttcctgagcctcacctgtcttggctggaaaacggcgaggaactgaacgccatcaacaccaccgtgtctcaggaccccgaaaccgagctgtacgctgtgtcctccaagctggacttcaacatgaccaccaaccacagcttcatgtgcctgattaagtacggccacctgagagtgaaccagaccttcaactggaacaccaccaagcaagagcacttccctgacaatggatctggcggcggaggttctggcggaggtggaagcggaggcggaggatctgctgagtctaagtatggccctccttgtcctccatgtcctgctccagaagctgctggcggaccctctgtgttcctgtttcctccaaagcctaaggaccagctcatgatctctcggacacccgaagtgacctgcgtggtggtggatgtgtctcaagaggaccctgaggtgcagttcaattggtacgtggacggcgtggaagtgcacaacgccaagaccaagcctagagaggaacagttcaactccacctacagagtggtgtccgtgctgaccgtgctgcaccaggattggctgaacggcaaagagtacaagtgcaaggtgtccaacaagggcctgccttccagcatcgaaaagaccatctccaaggctaagggccagcctagggaaccccaggtttacaccctgcctccaagccaagaggaaatgaccaagaaccaggtgtccctgacctgcctggtcaagggcttctacccttccgacattgccgtggaatgggagtccaatggccagcctgagaacaactacaagaccacacctcctgtgctggactccgacggctccttctttctgtactctcgcctgaccgtggacaagtctagatggcaagagggcaacgtgttctcctgctctgtgctgcacgaggccctgcacaatcactacacccagaagtccctgtctctgtctcttggaggtggtggcggttctgcccctaccagctcctctaccaagaaaacccagctccagttggagcatctgctgctggacctccagatgattctgaacgggatcaacaactataagaaccccaagctgaccgccatgctgaccgctaagttctacatgcccaagaaggccaccgagctgaagcacctccagtgcctggaaagggaactgaagcccctggaagaggtgctgaatctggcccagtccaagaacttccacctgaggccacgggacctgatcagcaacatcaacgtgatcgtgctggaactgaagggctccgagacaacctttatgtgcgagtacgccgacgagacagccaccatcgtggaatttctgaaccggtggatcaccttctgccagagcatcatctccacactgacc

SEQ ID NO: 28 - protein, 592 aa, Artificial Sequence
  fusion protein (GI102-M61)
VIHVTKEVKEVATLSCGHNVSVEELAQTRIYWQKEKKMVLTMMSGDMNIWPEYKNRTIFDITNNLSIVILALRPSDEGTYECVVLKYEKDAFKREHLAEVTLSVKADFPTPSISDFEIPTSNIRRIICSTSGGFPEPHLSWLENGEELNAINTTVSQDPETELYAVSSKLDFNMTTNHSFMCLIKYGHLRVNQTFNWNTTKQEHFPDNGSGGGGSGGGGSGGGGSAESKYGPPCPPCPAPEAAGGPSVFLFPPKPKDQLMISRTPEVTCVVVDVSQEDPEVQFNWYVDGVEVHNAKTKPREEQFNSTYRVVSVLTVLHQDWLNGKEYKCKVSNKGLPSSIEKTISKAKGQPREPQVYTLPPSQEEMTKNQVSLTCLVKGFYPSDIAVEWESNGQPENNYKTTPPVLDSDGSFFLYSRLTVDKSRWQEGNVFSCSVLHEALHNHYTQKSLSLSLGGGGGSAPTSSSTKKTQLQLEHLLLDLQMILNGINNYKNPKLTAMLTAKFYMPKKATELKHLQCLERELKPLEEVLNLAQSKNFHLRPRDLISNINVIVLELKGSETTFMCEYADETATIVEFLNRWITFCQSIISTLT

SEQ ID NO: 29 - DNA, 1857 bp, Artificial Sequence
  nucleotiedes coding fusion protein (GI102-M72)
atggatgctatgctgagaggcctgtgttgcgtgctgctgctgtgtggcgctgtgttcgtgtctccttctcacgctgtgatccacgtgaccaaagaagtgaaagaggtcgccacactgtcctgcggccacaacgtttcagtggaagaactggcccagaccaggatctactggcagaaagaaaagaaaatggtgctgaccatgatgtccggcgacatgaacatctggcctgagtacaagaaccggaccatcttcgacatcaccaacaacctgtccatcgtgattctggccctgaggccttctgatgagggcacctatgagtgcgtggtgctgaagtacgagaaggacgccttcaagcgcgagcacctggctgaagtgacactgtccgtgaaggccgactttcccacaccttccatctccgacttcgagatccctacctccaacatccggcggatcatctgttctacctctggcggctttcctgagcctcacctgtcttggctggaaaacggcgaggaactgaacgccatcaacaccaccgtgtctcaggaccccgaaaccgagctgtacgctgtgtcctccaagctggacttcaacatgaccaccaaccacagcttcatgtgcctgattaagtacggccacctgagagtgaaccagaccttcaactggaacaccaccaagcaagagcacttccctgacaatggatctggcggcggaggttctggcggaggtggaagcggaggcggaggatctgctgagtctaagtatggccctccttgtcctccatgtcctgctccagaagctgctggcggaccctctgtgttcctgtttcctccaaagcctaaggaccagctcatgatctctcggacacccgaagtgacctgcgtggtggtggatgtgtctcaagaggaccctgaggtgcagttcaattggtacgtggacggcgtggaagtgcacaacgccaagaccaagcctagagaggaacagttcaactccacctacagagtggtgtccgtgctgaccgtgctgcaccaggattggctgaacggcaaagagtacaagtgcaaggtgtccaacaagggcctgccttccagcatcgaaaagaccatctccaaggctaagggccagcctagggaaccccaggtttacaccctgcctccaagccaagaggaaatgaccaagaaccaggtgtccctgacctgcctggtcaagggcttctacccttccgacattgccgtggaatgggagtccaatggccagcctgagaacaactacaagaccacacctcctgtgctggactccgacggctccttctttctgtactctcgcctgaccgtggacaagtctagatggcaagagggcaacgtgttctcctgctctgtgctgcacgaggccctgcacaatcactacacccagaagtccctgtctctgtctcttggaggtggtggcggttctgcccctaccagctcctctaccaagaaaacccagctccagttggagcatctgctgctggacctccagatgattctgaacgggatcaacaactataagaaccccaagctgaccgccatgctgaccgctaagttctacatgcccaagaaggccaccgagctgaagcacctccagtgcctggaagaagaactgaagcccctggaagaggtgctgaatggggcccagtccaagaacttccacctgaggccacgggacctgatcagcaacatcaacgtgatcgtgctggaactgaagggctccgagacaacctttatgtgcgagtacgccgacgagacagccaccatcgtggaatttctgaaccggtggatcaccttctgccagagcatcatctccacactgacctgatga

SEQ ID NO: 30 - protein, 592 aa, Artificial Sequence
  fusion protein (GI102-M72)
VIHVTKEVKEVATLSCGHNVSVEELAQTRIYWQKEKKMVLTMMSGDMNIWPEYKNRTIFDITNNLSIVILALRPSDEGTYECVVLKYEKDAFKREHLAEVTLSVKADFPTPSISDFEIPTSNIRRIICSTSGGFPEPHLSWLENGEELNAINTTVSQDPETELYAVSSKLDFNMTTNHSFMCLIKYGHLRVNQTFNWNTTKQEHFPDNGSGGGGSGGGGSGGGGSAESKYGPPCPPCPAPEAAGGPSVFLFPPKPKDQLMISRTPEVTCVVVDVSQEDPEVQFNWYVDGVEVHNAKTKPREEQFNSTYRVVSVLTVLHQDWLNGKEYKCKVSNKGLPSSIEKTISKAKGQPREPQVYTLPPSQEEMTKNQVSLTCLVKGFYPSDIAVEWESNGQPENNYKTTPPVLDSDGSFFLYSRLTVDKSRWQEGNVFSCSVLHEALHNHYTQKSLSLSLGGGGGSAPTSSSTKKTQLQLEHLLLDLQMILNGINNYKNPKLTAMLTAKFYMPKKATELKHLQCLEEELKPLEEVLNGAQSKNFHLRPRDLISNINVIVLELKGSETTFMCEYADETATIVEFLNRWITFCQSIISTLT

SEQ ID NO: 31 - DNA, 1851 bp, Artificial Sequence
  nucleotiedes coding fusion protein (GI101w)
atggatgctatgctgagaggcctgtgttgcgtgctgctgctgtgtggcgctgtgttcgtgtctccttctcacgctgtgatccacgtgaccaaagaagtgaaagaggtcgccacactgtcctgcggccacaacgtttcagtggaagaactggcccagaccaggatctactggcagaaagaaaagaaaatggtgctgaccatgatgtccggcgacatgaacatctggcctgagtacaagaaccggaccatcttcgacatcaccaacaacctgtccatcgtgattctggccctgaggccttctgatgagggcacctatgagtgcgtggtgctgaagtacgagaaggacgccttcaagcgcgagcacctggctgaagtgacactgtccgtgaaggccgactttcccacaccttccatctccgacttcgagatccctacctccaacatccggcggatcatctgttctacctctggcggctttcctgagcctcacctgtcttggctggaaaacggcgaggaactgaacgccatcaacaccaccgtgtctcaggaccccgaaaccgagctgtacgctgtgtcctccaagctggacttcaacatgaccaccaaccacagcttcatgtgcctgattaagtacggccacctgagagtgaaccagaccttcaactggaacaccaccaagcaagagcacttccctgacaatggatctggcggcggaggttctggcggaggtggaagcggaggcggaggatctgctgagtctaagtatggccctccttgtcctccatgtcctgctccagaagctgctggcggaccctctgtgttcctgtttcctccaaagcctaaggaccagctcatgatctctcggacacccgaagtgacctgcgtggtggtggatgtgtctcaagaggaccctgaggtgcagttcaattggtacgtggacggcgtggaagtgcacaacgccaagaccaagcctagagaggaacagttcaactccacctacagagtggtgtccgtgctgaccgtgctgcaccaggattggctgaacggcaaagagtacaagtgcaaggtgtccaacaagggcctgccttccagcatcgaaaagaccatctccaaggctaagggccagcctagggaaccccaggtttacaccctgcctccaagccaagaggaaatgaccaagaaccaggtgtccctgacctgcctggtcaagggcttctacccttccgacattgccgtggaatgggagtccaatggccagcctgagaacaactacaagaccacacctcctgtgctggactccgacggctccttctttctgtactctcgcctgaccgtggacaagtctagatggcaagagggcaacgtgttctcctgctctgtgctgcacgaggccctgcacaatcactacacccagaagtccctgtctctgtctcttggaggtggtggcggttctgcccctaccagctcctctaccaagaaaacccagctccagttggagcatctgctgctggacctccagatgattctgaacgggatcaacaactataagaaccccaagctgacccgcatgctgacctttaagttctacatgcccaagaaggccaccgagctgaagcacctccagtgcctggaagaagaactgaagcccctggaagaggtgctgaatctggcccagtccaagaacttccacctgaggccacgggacctgatcagcaacatcaacgtgatcgtgctggaactgaagggctccgagacaacctttatgtgcgagtacgccgacgagacagccaccatcgtggaatttctgaaccggtggatcaccttctgccagagcatcatctccacactgacc

SEQ ID NO: 32 - protein, 592 aa, Artificial Sequence
  fusion protein (GI101w)
VIHVTKEVKEVATLSCGHNVSVEELAQTRIYWQKEKKMVLTMMSGDMNIWPEYKNRTIFDITNNLSIVILALRPSDEGTYECVVLKYEKDAFKREHLAEVTLSVKADFPTPSISDFEIPTSNIRRIICSTSGGFPEPHLSWLENGEELNAINTTVSQDPETELYAVSSKLDFNMTTNHSFMCLIKYGHLRVNQTFNWNTTKQEHFPDNGSGGGGSGGGGSGGGGSAESKYGPPCPPCPAPEAAGGPSVFLFPPKPKDQLMISRTPEVTCVVVDVSQEDPEVQFNWYVDGVEVHNAKTKPREEQFNSTYRVVSVLTVLHQDWLNGKEYKCKVSNKGLPSSIEKTISKAKGQPREPQVYTLPPSQEEMTKNQVSLTCLVKGFYPSDIAVEWESNGQPENNYKTTPPVLDSDGSFFLYSRLTVDKSRWQEGNVFSCSVLHEALHNHYTQKSLSLSLGGGGGSAPTSSSTKKTQLQLEHLLLDLQMILNGINNYKNPKLTRMLTFKFYMPKKATELKHLQCLEEELKPLEEVLNLAQSKNFHLRPRDLISNINVIVLELKGSETTFMCEYADETATIVEFLNRWITFCQSIISTLT

SEQ ID NO: 33 - DNA, 1848 bp, Artificial Sequence
  nucleotiedes coding fusion protein (mGI102-M61)
atggatgctatgctgagaggcctgtgttgcgtgctgctgctgtgtggcgctgtgttcgtgtctccttctcacgctgtggacgagcagctctccaagtccgtgaaggataaggtcctgctgccttgccggtacaactctcctcacgaggacgagtctgaggaccggatctactggcagaaacacgacaaggtggtgctgtccgtgatcgccggaaagctgaaagtgtggcctgagtacaagaacaggaccctgtacgacaacaccacctacagcctgatcatcctgggcctcgtgctgagcgatagaggcacctattcttgcgtggtgcagaagaaagagcggggcacctacgaagtgaagcacctggctctggtcaagctgtccatcaaggccgacttcagcacccctaacatcaccgagtctggcaacccttccgccgacaccaagagaatcacctgtttcgcctctggcggcttccctaagcctcggttctcttggctggaaaacggcagagagctgcccggcatcaataccaccatttctcaggacccagagtccgagctgtacaccatctccagccagctcgactttaacaccaccagaaaccacaccatcaagtgcctgattaagtacggcgacgcccacgtgtccgaggactttacttgggagaaacctcctgaggaccctcctgactctggatctggcggcggaggttctggcggaggtggaagcggaggcggaggatctgctgagtctaagtatggccctccttgtcctccatgtcctgctccagaagctgctggcggaccctctgtgttcctgtttcctccaaagcctaaggaccagctcatgatctctcggacccctgaagtgacctgcgtggtggtggatgtgtctcaagaggaccctgaggtgcagttcaattggtacgtggacggcgtggaagtgcacaacgccaagaccaagcctagagaggaacagttcaactccacctatagagtggtgtccgtgctgaccgtgctgcaccaggattggctgaacggcaaagagtacaagtgcaaggtgtccaacaagggcctgccttccagcatcgaaaagaccatcagcaaggctaagggccagcctagggaaccccaggtttacaccctgcctccaagccaagaggaaatgaccaagaaccaggtgtccctgacctgcctggtcaagggcttctacccttccgacattgccgtggaatgggagtccaatggccagcctgagaacaactacaagaccacacctcctgtgctggactccgacggctccttctttctgtactctcgcctgaccgtggacaagtctaggtggcaagagggcaacgtgttctcctgctctgtgctgcacgaggctctgcacaaccactacacccagaagtccctgtctctgtctcttggaggtggtggcggttctgcccctacctccagctctaccaagaaaacccagctccagttggagcatctgctgctggacctccagatgatcctgaatggcatcaacaattacaagaaccccaagctgaccgccatgctgaccgctaagttctacatgcccaagaaggccaccgagctgaagcacttgcagtgcctggaaagggaactgaagcccctggaagaagtgctgaatctggcccagtccaagaacttccacctgaggcctagggacctgatctccaacatcaacgtgatcgtgctggaactgaaaggctccgagacaaccttcatgtgcgagtacgccgacgagacagccaccatcgtggaatttctgaaccggtggatcaccttctgccagagcatcatctccacactgacc

SEQ ID NO: 34 - protein, 616 aa, Artificial Sequence
  fusion protein (mGI102-M61)
MDAMLRGLCCVLLLCGAVFVSPSHAVDEQLSKSVKDKVLLPCRYNSPHEDESEDRIYWQKHDKVVLSVIAGKLKVWPEYKNRTLYDNTTYSLIILGLVLSDRGTYSCVVQKKERGTYEVKHLALVKLSIKADFSTPNITESGNPSADTKRITCFASGGFPKPRFSWLENGRELPGINTTISQDPESELYTISSQLDFNTTRNHTIKCLIKYGDAHVSEDFTWEKPPEDPPDSGSGGGGSGGGGSGGGGSAESKYGPPCPPCPAPEAAGGPSVFLFPPKPKDQLMISRTPEVTCVVVDVSQEDPEVQFNWYVDGVEVHNAKTKPREEQFNSTYRVVSVLTVLHQDWLNGKEYKCKVSNKGLPSSIEKTISKAKGQPREPQVYTLPPSQEEMTKNQVSLTCLVKGFYPSDIAVEWESNGQPENNYKTTPPVLDSDGSFFLYSRLTVDKSRWQEGNVFSCSVLHEALHNHYTQKSLSLSLGGGGGSAPTSSSTKKTQLQLEHLLLDLQMILNGINNYKNPKLTAMLTAKFYMPKKATELKHLQCLERELKPLEEVLNLAQSKNFHLRPRDLISNINVIVLELKGSETTFMCEYADETATIVEFLNRWITFCQSIISTLT

SEQ ID NO: 35 - protein, 153 aa, Artificial Sequence
  wild type hIL-2
MYRMQLLSCIALSLALVTNSAPTSSSTKKTQLQLEHLLLDLQMILNGINNYKNPKLTRMLTFKFYMPKKATELKHLQCLEEELKPLEEVLNLAQSKNFHLRPRDLISNINVIVLELKGSETTFMCEYADETATIVEFLNRWITFCQSIISTLT

SEQ ID NO: 36 - protein, 158 aa, Artificial Sequence
  IL-2 with signal sequence
MDAMLRGLCCVLLLCGAVFVSPSHAAPTSSSTKKTQLQLEHLLLDLQMILNGINNYKNPKLTRMLTFKFYMPKKATELKHLQCLEEELKPLEEVLNLAQSKNFHLRPRDLISNINVIVLELKGSETTFMCEYADETATIVEFLNRWITFCQSIISTLT

SEQ ID NO: 37 - DNA, 474 bp, Artificial Sequence
  nucleotide sequence coding IL-2 with signal sequence
atggatgctatgctgagaggcctgtgttgcgtgctgctgctgtgtggcgctgtgttcgtgtctccttctcacgctgcccctaccagctcctctaccaagaaaacccagctccagttggagcatctgctgctggacctccagatgattctgaacgggatcaacaactataagaaccccaagctgacccgcatgctgacctttaagttctacatgcccaagaaggccaccgagctgaagcacctccagtgcctggaagaagaactgaagcccctggaagaggtgctgaatctggcccagtccaagaacttccacctgaggccacgggacctgatcagcaacatcaacgtgatcgtgctggaactgaagggctccgagacaacctttatgtgcgagtacgccgacgagacagccaccatcgtggaatttctgaaccggtggatcaccttctgccagagcatcatctccacactgacc

SEQ ID NO: 38 - protein, 591 aa, Artificial Sequence
  mGI-101
VDEQLSKSVKDKVLLPCRYNSPHEDESEDRIYWQKHDKVVLSVIAGKLKVWPEYKNRTLYDNTTYSLIILGLVLSDRGTYSCVVQKKERGTYEVKHLALVKLSIKADFSTPNITESGNPSADTKRITCFASGGFPKPRFSWLENGRELPGINTTISQDPESELYTISSQLDFNTTRNHTIKCLIKYGDAHVSEDFTWEKPPEDPPDSGSGGGGSGGGGSGGGGSAESKYGPPCPPCPAPEAAGGPSVFLFPPKPKDQLMISRTPEVTCVVVDVSQEDPEVQFNWYVDGVEVHNAKTKPREEQFNSTYRVVSVLTVLHQDWLNGKEYKCKVSNKGLPSSIEKTISKAKGQPREPQVYTLPPSQEEMTKNQVSLTCLVKGFYPSDIAVEWESNGQPENNYKTTPPVLDSDGSFFLYSRLTVDKSRWQEGNVFSCSVLHEALHNHYTQKSLSLSLGGGGGSAPTSSSTKKTQLQLEHLLLDLQMILNGINNYKNPKLTAMLTAKFYMPKKATELKHLQCLEEELKPLEEVLNLAQSKNFHLRPRDLISNINVIVLELKGSETTFMCEYADETATIVEFLNRWITFCQSIISTLT